European Patent Application EP 4 803 903 A1, published September 9, 2026. Title: An improved quantitative immunoassay for the detection of autoantibodies to nephrin. Applicant: EUROIMMUN Medizinische Labordiagnostika AG. Application EP. The sequence listing filed with the application follows.

SEQUENCE LISTING (29 sequences)

SEQ ID NO: 1 - protein, 1055 aa, synthetic construct
  source 1..1055: note = consensus sequence
  SITE 15: note = G or E
  SITE 16: note = M or L
  SITE 18: note = T or M
  SITE 28: note = T or A
  SITE 38: note = S or P
  SITE 39: note = E or A
  SITE 41: note = L or M
  SITE 43: note = V or A
  SITE 49: note = V or A
  SITE 50: note = K or E
  SITE 61: note = V or A
  SITE 74: note = N or D
  SITE 75: note = P or R
  SITE 76: note = K or R
  SITE 77: note = I or M
  SITE 91: note = K or R
  SITE 100: note = A or E
  SITE 114: note = G or S
  SITE 128: note = I or V
  SITE 130: note = S or T
  SITE 131: note = I or V
  SITE 134: note = S or P
  SITE 137: note = V or L
  SITE 139: note = Q or L
  SITE 146: note = S or T
  SITE 147: note = T or M
  SITE 163: note = G or P
  SITE 170: note = D or E
  SITE 173: note = F or I
  SITE 175: note = Q or L
  SITE 179: note = T or V
  SITE 180: note = V or I
  SITE 182: note = D or G
  SITE 183: note = V or I
  SITE 185: note = S or A
  SITE 186: note = S or N
  SITE 193: note = E or Q
  SITE 196: note = F or C
  SITE 198: note = T or V
  SITE 202: note = A or V
  SITE 205: note = T or I
  SITE 207: note = Q or R
  SITE 212: note = G or R
  SITE 213: note = Q or K
  SITE 221: note = N or S
  SITE 226: note = T or A
  SITE 228: note = I or L
  SITE 229: note = K or R
  SITE 230: note = A or V
  SITE 232: note = F or V
  SITE 234: note = M or V
  SITE 236: note = I or V
  SITE 238: note = F or C
  SITE 239: note = P or K
  SITE 240: note = P or W
  SITE 241: note = G or absent
  SITE 243: note = P or absent
  SITE 245: note = I or absent
  SITE 247: note = W or R
  SITE 248: note = P or T
  SITE 249: note = G or E
  SITE 251: note = N or D
  SITE 254: note = H or Q
  SITE 259: note = E or Q
  SITE 267: note = A or S
  SITE 273: note = P or L
  SITE 283: note = K or Q
  SITE 287: note = I or T
  SITE 296: note = A or S
  SITE 299: note = H or R
  SITE 307: note = R or W
  SITE 313: note = A or V
  SITE 314: note = R or Q
  SITE 318: note = Q or E
  SITE 319: note = S or A
  SITE 325: note = A or T
  SITE 327: note = T or I
  SITE 328: note = Q or R
  SITE 331: note = S or G
  SITE 332: note = I or V
  SITE 333: note = T or M
  SITE 343: note = V or I
  SITE 344: note = T or I
  SITE 352: note = S or T
  SITE 359: note = L or V
  SITE 360: note = C or S
  SITE 363: note = T or S
  SITE 373: note = R or Q
  SITE 378: note = G or W
  SITE 385: note = D or E
  SITE 386: note = E or D
  SITE 387: note = T or M
  SITE 389: note = M or V
  SITE 393: note = H or Y
  SITE 406: note = V or A
  SITE 407: note = K or R
  SITE 422: note = D or E
  SITE 425: note = S or T
  SITE 432: note = S or T
  SITE 434: note = T or I
  SITE 436: note = N or S
  SITE 451: note = E or V
  SITE 455: note = I or L
  SITE 457: note = T or A
  SITE 459: note = T or N
  SITE 464: note = V or M
  SITE 473: note = E or D
  SITE 481: note = D or A
  SITE 487: note = D or E
  SITE 488: note = P or S
  SITE 491: note = S or P
  SITE 494: note = P or S
  SITE 498: note = Q or H
  SITE 502: note = V or L
  SITE 508: note = T or I
  SITE 514: note = V or I
  SITE 516: note = I or V
  SITE 517: note = I or T
  SITE 520: note = P or S
  SITE 525: note = K or T
  SITE 527: note = S or T
  SITE 538: note = Q or R
  SITE 539: note = L or F
  SITE 540: note = V or A
  SITE 548: note = L or V
  SITE 554: note = S or A
  SITE 555: note = S or T
  SITE 556: note = A or T
  SITE 561: note = D or E
  SITE 568: note = V or I
  SITE 570: note = I or V
  SITE 577: note = N or S
  SITE 580: note = L or W
  SITE 586: note = R or G
  SITE 588: note = D or E
  SITE 594: note = P or A
  SITE 595: note = Q or R
  SITE 600: note = K or R
  SITE 605: note = S or A
  SITE 607: note = S or T
  SITE 609: note = F or L
  SITE 611: note = R or Q
  SITE 613: note = S or T
  SITE 614: note = S or P
  SITE 619: note = H or Q
  SITE 620: note = R or H
  SITE 624: note = R or S
  SITE 631: note = R or Q
  SITE 634: note = V or M
  SITE 636: note = S or A
  SITE 640: note = L or F
  SITE 645: note = P or R
  SITE 654: note = R or L
  SITE 658: note = V or A
  SITE 661: note = Q or K
  SITE 663: note = Q or E
  SITE 664: note = A or V
  SITE 671: note = S or absent
  SITE 672: note = A or absent
  SITE 673: note = N or S
  SITE 681: note = W or G
  SITE 701: note = G or S
  SITE 705: note = Q or H
  SITE 707: note = W or S
  SITE 714: note = D or G
  SITE 716: note = F or L
  SITE 730: note = A or T
  SITE 731: note = L or R
  SITE 732: note = L or V
  SITE 733: note = K or R
  SITE 737: note = H or Q
  SITE 741: note = T or A
  SITE 742: note = I or V
  SITE 744: note = A or V
  SITE 752: note = N or D
  SITE 753: note = V or I
  SITE 759: note = I or L
  SITE 780: note = E or G
  SITE 781: note = D or E
  SITE 784: note = E or D
  SITE 786: note = N or S
  SITE 792: note = K or M
  SITE 795: note = K or R
  SITE 797: note = S or P
  SITE 802: note = R or Q
  SITE 805: note = Q or H
  SITE 807: note = K or E
  SITE 817: note = I or V
  SITE 818: note = V or A
  SITE 825: note = A or P
  SITE 828: note = G or R
  SITE 830: note = V or L
  SITE 836: note = F or Y
  SITE 839: note = Q or H
  SITE 841: note = D or E
  SITE 842: note = H or Q
  SITE 844: note = T or A
  SITE 867: note = G or A
  SITE 871: note = I or V
  SITE 872: note = D or V
  SITE 881: note = P or A
  SITE 885: note = Q or E
  SITE 899: note = V or I
  SITE 907: note = A or T
  SITE 913: note = Q or H
  SITE 919: note = K or T
  SITE 921: note = T or I
  SITE 925: note = A or P
  SITE 931: note = T or I
  SITE 949: note = V or A
  SITE 950: note = V or M
  SITE 953: note = S or T
  SITE 982: note = S or T
  SITE 986: note = L or H
  SITE 987: note = Y or H
  SITE 988: note = M or V
  SITE 991: note = L or V
  SITE 994: note = Q or D
  SITE 1004: note = K or Q
  SITE 1032: note = S or P
  SITE 1038: note = L or P
  SITE 1039: note = D or H
  SITE 1041: note = A or P
  SITE 1042: note = P or S
  SITE 1045: note = T or P
  SITE 1048: note = P or Q
  SITE 1049: note = L or P
XXXXXXXXXXLLLXXXLXXGLXXXXXXXSXPRGFWALXXNXTXVEGXXXXLXCGVXXPGSXVQWAKDGLLLGPXXXXPXFPRYXLEGDXXXGEFHLXIEXCDLSDDAEYECQVXRSEXGPELVSPXVXLXXLVXPKXLXLTPEAGXXVTWVAGQEYXVXCVSXDAKPAPXIXXXXXGXXXXXXSXXVNXGSXXKLXXXEAXXRVXPXSSDNXXLLVCEXSXPALXXPXXXSXTXNXLXXXXXXXXXXXXLXEGXVRAGXXLELXCXXRGGNPXATLQWLKNGXPXSXAWGTEHXXXVAXSXLVMXVXPEDHGXXLSCXXXNSVSXXXXEXXXXLQVTFPPSAXXILGSXSQXENKNVTXXCXXKSSRPRVLLXWWLGXRQLXPXXXXVXDGLXGGHISMSNLTXLXXREDNGLXLTCEAFSXAFXKETFKKXLXLXVKYPAQKLWIEGPPXGQXXRXGXRVRLXCLAIGGNPXPXLXWXKXSRXVXXXRXXQEXRRVXLGSXEKSGSXFSRELXLXXGPXDNXAXFXCKAGQLSASTXXXVQFPPTNXTILANXXXLRPGXALNLTCXSXSSNPPVXLSXDKEGEXLXXVAXXXXXAPFXGSAAXRXVXLXXXXRDHGXXVTCXAHSXXLXETXSXFYRXNVLYXPEFLGEQVXXVTXVEXGXXLLPVSVXXXPAPEAFNXTFRGYRLSPAGGPRHRILSXGALXLXNVTRADXGXYQLHCQNSEGTAEXXXXLDVXYAPXXRXLXDPTEVXXGXSVDXVCTVDANPILPXMFXWERLGXXXEXXXLDDMEXXSXGXTGRLXIXXAXLXQAGAYQCXXDNGVAPXARXLXRLVVRXAPXVXXPXPLXKVAAAGDSTSSATLHCRARXVPNXXFTWXKNGVXLDLXDPRYTEHXYHQGXXHSSLLTIXNVSAAXDYALFXCXATNXLGSDXXNIQLVSISRPDPPXGLKXXSXXPXSVGLEWKPGFDGGLPQXFXIRYEALXXPGFXXXDVXPXXATXFTLTGLXPSTRYRXWLLASNALGDSGLXDKGXQXXXTTPGXXXXXXXXXXXXPTEXPX

SEQ ID NO: 2 - protein, 1055 aa, synthetic construct
  source 1..1055: note = extracellular domain of human nephrin
MALGTTLRASLLLLGLLTEGLAQLAIPASVPRGFWALPENLTVVEGASVELRCGVSTPGSAVQWAKDGLLLGPDPRIPGFPRYRLEGDPARGEFHLHIEACDLSDDAEYECQVGRSEMGPELVSPRVILSILVPPKLLLLTPEAGTMVTWVAGQEYVVNCVSGDAKPAPDITILLSGQTISDISANVNEGSQQKLFTVEATARVTPRSSDNRQLLVCEASSPALEAPIKASFTVNVLFPPGPPVIEWPGLDEGHVRAGQSLELPCVARGGNPLATLQWLKNGQPVSTAWGTEHTQAVARSVLVMTVRPEDHGAQLSCEAHNSVSAGTQEHGITLQVTFPPSAIIILGSASQTENKNVTLSCVSKSSRPRVLLRWWLGWRQLLPMEETVMDGLHGGHISMSNLTFLARREDNGLTLTCEAFSEAFTKETFKKSLILNVKYPAQKLWIEGPPEGQKLRAGTRVRLVCLAIGGNPEPSLMWYKDSRTVTESRLPQESRRVHLGSVEKSGSTFSRELVLVTGPSDNQAKFTCKAGQLSASTQLAVQFPPTNVTILANASALRPGDALNLTCVSVSSNPPVNLSWDKEGERLEGVAAPPRRAPFKGSAAARSVLLQVSSRDHGQRVTCRAHSAELRETVSSFYRLNVLYRPEFLGEQVLVVTAVEQGEALLPVSVSANPAPEAFNWTFRGYRLSPAGGPRHRILSSGALHLWNVTRADDGLYQLHCQNSEGTAEARLRLDVHYAPTIRALQDPTEVNVGGSVDIVCTVDANPILPGMFNWERLGEDEEDQSLDDMEKISRGPTGRLRIHHAKLAQAGAYQCIVDNGVAPPARRLLRLVVRFAPQVEHPTPLTKVAAAGDSTSSATLHCRARGVPNIVFTWTKNGVPLDLQDPRYTEHTYHQGGVHSSLLTIANVSAAQDYALFTCTATNALGSDQTNIQLVSISRPDPPSGLKVVSLTPHSVGLEWKPGFDGGLPQRFCIRYEALGTPGFHYVDVVPPQATTFTLTGLQPSTRYRVWLLASNALGDSGLADKGTQLPITTPGLHQPSGEPEDQLPTEPPS

SEQ ID NO: 3 - protein, 1078 aa, synthetic construct
  source 1..1078: note = extracellular domain of murine nephrin
MGAKEATVRGPGASPVHRTCHLIPLLLAGMLTTGLAQSPVPTSAPRGFWALSENLTVVEGSTVKLWCGVRAPGSVVQWAKDGLLLGPNPKIPGFPRYSLEGDSAKGEFHLLIEACDLSDDAEYECQVGRSELGPELVSPSVILSILVSPKVLQLTPEAGSTVTWVAGQEYVVTCVSGDAKPAPDIIFIQGGRTVEDVSSSVNEGSEEKLFFTEAEARVTPQSSDNGQLLVCEGSNPALATPIKASFTMNILFPPGPPVIDWPGLNEGHVRAGENLELPCIARGGNPPATLQWLKNGKPVSIAWGTEHAQAVAHSVLVMTVRPEDHGARLSCQSYNSVSAETQERSITLQVTFPPSAVTILGSTSQSENKNVTLCCLTKSSRPRVLLRWWLGGRQLLPTDETVMDGLHGGHISMSNLTLLVKREDNGLSLTCEAFSDAFSKETFKKSLTLNVKYPAQKLWIEGPPEGQSIRTGTRVRLVCLAIGGNPEPSLTWLKDSRPVNDPRQSQEPRRVQLGSVEKSGSTFSRELVLIIGPPDNLAKFSCKAGQLSASTQLVVQFPPTNLTILANSSALRPGDALNLTCVSISSNPPVNLSLDKEGERLDDVAAKPQSAPFKGSAASRSVFLRVSSRDHGHRVTCRAHSEALRETVSSFYRLNVLYPPEFLGEQVRAVTVVEQGQALLPVSVSANPAPEAFNWTFRGYRLSPAGGPRHRILSGGALQLWNVTRADDGFYQLHCQNSEGTAEALLKLDVHYAPTIRALKDPTEVNVGGSVDIVCTVDANPILPEMFSWERLGEDEEELNLDDMEKMSKGSTGRLRIRQAKLSQAGAYQCIVDNGVAPAARGLVRLVVRFAPQVDHPTPLTKVAAAGDSTSSATLHCRARGVPNIDFTWTKNGVPLDLQDPRYTEHKYHQGVVHSSLLTIANVSAAQDYALFKCTATNALGSDHTNIQLVSISRPDPPLGLKVVSVSPHSVGLEWKPGFDGGLPQRFQIRYEALESPGFLYMDVLPAQATTFTLTGLKPSTRYRIWLLASNALGDSGLTDKGIQVSITTPGLDQAPEDTDQPLPTEQPPGPPRLPLLP

SEQ ID NO: 4 - protein, 1078 aa, synthetic construct
  source 1..1078: note = extracellular domain of rat nephrin
MGAKRVTVRGARTSPIHRMSSLTPLLLMGMLTSGLAESPVPTSAPRGFWALSENLTAVEGTTVKLWCGVRAPGSVVQWAKDGLLLGPNPKMPGFPRYSLEGDRAKGEFHLLIEACDLSDDAEYECQVGRSELGPELVSPKVILSILVSPKVLLLTPEAGSTVTWVAGQEYVVTCVSGDAKPAPDITFIQSGRTILDVSSNVNEGSEEKLCITEAEARVIPQSSDNGQLLVCEGSNPALDTPIKASFTMNILFPPGPPVIDWPGLNEGHVRAGENLELPCTARGGNPPATLQWLKNGKPVSTAWGTEHAQAVAHSVLVMTVRPEDHGARLSCQSYNSVSAGTQERSITLQVTFPPSAITILGSVSQSENKNVTLCCLTKSSRPRVLLRWWLGGRQLLPTDETVMDGLHGGHISMSNLTFLVRREDNGLPLTCEAFSDAFSKETFKKSLTLNVKYPAQKLWIEGPPEGQYIRTGTRVRLVCLAIGGNPDPSLIWFKDSRPVSEPRQPQEPRRVQLGSVEKSGSTFSRELVLIIGPPDNRAKFSCKAGQLSASTQLVVQFPPTNLTILANSSALRPGDALNLTCVSISSNPPVNLSWDKEGERLEDVAAKPQSAPFKGSAASRSVFLRVSSRDHGQRVTCRAHSEALRETVSSFYRFNVLYPPEFLGEQVRAVTVVEQGQVLLPVSVSANPAPEAFNWTFRGYRLSPAGGPRHRILSGGALQLWNVTRADDGFYQLHCQNSEGTAEALLKLDVHYAPTIRALRDPTEVNVGGSVDIVCTVDANPILPEMFSWERLGEEEEDLNLDDMEKVSKGSTGRLRIRQAKLSQAGAYQCIVDNGVAPAARGLVRLVVRFAPQVDQPTPLTKVAAAGDSTSSATLHCRARGVPNIDFTWTKNGVPLDLQDPRYTEHRYHQGVVHSSLLTIANVSAAQDYALFKCTATNALGSDHTNIQLVSISRPDPPLGLKVVSISPHSVGLEWKPGFDGGLPQRFQIRYEALETPGFLHVDVLPTQATTFTLTGLKPSTRYRIWLLASNALGDSGLTDKGIQVSVTTPGPDQAPEDTDHQLPTELPPGPPRLPLLP

SEQ ID NO: 5 - protein, 1070 aa, synthetic construct
  source 1..1070: note = extracellular domain of rabbit nephrin
MTEPPRGLEVALRTPIGDALLLMGLLTTGLVQSSVPASAPRGFWALPANLTAVEGAEAELQCGVSAPGSAVQWAKDGLLLGPDPRIPGFPRYRLEGDPAKGEFHLHIEACDLSDDAEYECQVGRSEMGPELVSPRVVLSILVPPKVLQLTPEAGSTVTWVAGQEYVVSCVSPDAKPAPEITFLQSGQTVSDISANVNDGSQEKLFTTEATARVIPQSSDNGQLLVCESSSPALDTPLRASVTMNVLFPPGAPVIEWPGLNEGHVRAGQSLELPCVARGGNPPATLQWLKNGQPLSTAWGTEHVQAVARSVLVMTVWPEDHGARLSCEASNSVSAGTREQSVTLQVTFPPSAITILGSASQSENKNVTLSCITKSSRPRVLLQWWLGGRQLLPTEETVMDGLHGGHISMSNLTYLVRREDNGLTLTCEAFSEAFTKETFKKSLTLSVKYPAQKLWIEGPPEGQLLRTGTRVRLMCLAIGGNPDPALTWLKDSRTVTEPRLPQEPRRVQLGSLEKSGSTFSRELVLVIGPSDNKATFTCKAGQLSASTRLVVQFPPTNLTILANASALRPGDALNLTCISISSNPPVNLSWDKEGEGLESVAGLPQKAPFKGSAAARSVFLRVTSRDHGHHVTCRAHSAELRETVSSFYRLNVLYPPEFLGEQVLEVTAVEQGEALLPVSVSANPAPEAFNWTFRGYRLSPAGGPRHRILSSGALQLWNVTRADGGLYQLHCQNSEGTAEALVRLDVHYAPIIRALQDPTEVDVGGSVDLVCTVDANPILPDMFSWERLGEEEEDQSLDDMEKISKGSTGRLRILHAELAQAGAYQCVVDNGVAPPARGLVRLVVRYAPQVEHPAPLTKVAAAGDSTSSATLHCRARAVPNVVFTWTKNGVPLDLQDPRYTEHTYHQGGVHSSLLTIANVSAAHDYALFTCTATNPLGSDQTNIQLVSISRPDPPSGLKVVSLTPHSVGLEWKPGFDGGLPQKFRIRYEALDTPGFLYMDVLPAQATAFTLTGLQPSTRYRLWLLASNALGDSGLADKGIQLSLTTPGLDHPSGIPDHQPPTEQPAGPPGLR

SEQ ID NO: 6 - protein, 1061 aa, synthetic construct
  source 1..1061: note = extracellular domain of dog nephrin
MALRTPSRAPLLLMGLLTTGLAQLPLSASAPRGFWALPENLTVVEGATAELQCGVHAPGSVVQWAKDGLLLGPDPRIPRFPRYRLEGDPSRGEFHLHIEACDLSDDAEYECQVGRSETGPELVSPRVILSVLVPPKVLQLTPEAGSTVTWVAGQEYVVTCVSGDAKPAPDITFFQSGQTVSDISANVNAGSQEKLFTTEATARVTPQSSDNGQLLVCEGSSPALDTPIRVSVTMNVLFPPGPPVIEWPGLDEGHVRAGQSLELLCVARGGNPPATLQWLKNGQPMSTAWGTEHAEAVARSMLVMVVRPEDHGARLSCEAHNSVSTGIQERGVTLQVTFPPSAITILGSASQSENKNVTLSCISKSSRPRVLLRWWLGWRQLVPTEEMVVDGLHGGHISMSNLTFLVRREDNGLTLTCEAFSEAFTKETFKKSLTLNVKYPAQKLWIEGPPEGQRLRAGTRVRLVCLAIGGNPEPSLTWLKDSRTVTEPRPPQEPRRVQLGSLEKSGSTFSRELILITGPSDNQAKFTCKAGQLSASTQLVVQFPPTNVTILANATALRPGDALNLTCISVSSNPPVNLSWDKEGERLESVATPPRSAPFKGSAAARSVLLRMSSRDHGHRVTCRAHSPELRETMSAFYRLNVLYPPEFLGEQVLVVTAVEQGEALLPVSVSANPAPEAFNWTFRGYRLSPAGGPRHRILSGGALQLWNVTRADDGLYQLHCQNSEGTAETLVRLDVHYAPTIRALQDPTEVNIGGSVDIVCTVDANPILPEMFSWERLGEEEEDQSLDDMEKISKGSTGRLRIHHAKLAQAGAYQCIVDNGVAPPARGLVRLVVRFAPQVEHPTPLNKVAAAGDSTSSATLHCRARGVPNIVFTWAKNGVPLDLEDPRYTEHTYHQGGVHSSLLTIANVSAAQDYALFTCTATNPLGSDHTNIQLVSISRPDPPTGLKVVSMTPYSVGLEWKPGFDGGLPQKFQIRYEALGTPGFLYMDVLPPDATTFTLTGLQPSTRYRVWLLASNALGDSGLTDKGSQIPITTPGLDEPSGEPDYQLPTEQPVGPSGLP

SEQ ID NO: 7 - protein, 1055 aa, synthetic construct
  source 1..1055: note = extracellular domain of cat nephrin
MALRTPGRVPLLLLGLLTTGLARLPLPASTPRGFWALPENLTVVEGATAELRCGVSAPGSAVQWAKDGLLLGPDPRIPSFPRYRLEGDPDRGEFHLHIEACDLSDDAEYECQVGRSETGPELVSPRVILTILVPPKVLQLTPEAGSTVTWVAGQEYVVSCVSGDAKPAPDITFIQSGQTISDISANVNVGSQEKLFTTEATARVTPQSSDNGKLLVCEGSSPALDTPIRVSVTMNVLFPPGPPVIEWPGLDEGHVRAGQSLELLCVSRGGNPPATLQWLKNGQPVSTAWGTEHAEAVARSMLVMIVRPEDHGARLSCEAHNSVSTGIQERGVTLQVTFPPSAITILGSASQSENKNVTLSCITKSSRPRVLLRWWLGWRQLLPTEDMVMDGLHGGHISMSNLTFLVRREDNGLTLTCEAFSEAFTKETFKKSLILNVKYPAQKLWIEGPPEGQRLRAGTRVRLVCLAIGGNPDPSLTWFKDSRAVTEPRPPQEPRRVQLGSLEKSGSTFSRELVLITGPSDNQAKFTCKAGQLSASTQLVVQFPPTNVTILANASALRPGDALNLTCVSVSSNPPVNLSWDKEGERLESVAIPPRSAPFKGSAAARSVLLRMSSRDHGHRVTCRAHSTELRETMSAFYRLNVLYPPEFLGEQVLVVTAVEQGEALLPVSVSANPAPEAFNWTFRGYRLSPAGGPRHRILSGGALQLWNVTRADDGLYQLHCQNSEGTAEALVRLDVHYAPTIRVLQDPTEVNIGGSVDIVCTVDANPILPGMFNWERLGGEEEDHSLDDMEKMSKGSTGRLRIHHAKLDQAGAYQCIVDNGVAPPARGLVRLVVRFAPQVEHPTPLTKVAAAGDSTSSATLHCRARGVPNIVFTWTKNGVALDLQDPRYTEHTYHQGMVHSSLLTIANVSAAQDYALFTCTATNPLGSDRTNIQLVSISRPDPPTGLKVMSMTPYSVGLEWKPGFDGGLPQRFQIRYEALGTPGFLYMDVLPPQATTFTLTGLQPSTRYRVWLLASNALGDSGLMDKGSQISVTTPGLDQPSGEPDYQLPTEQPT

SEQ ID NO: 8 - protein, 1127 aa, synthetic construct
  source 1..1127: note = extracellular domain of equine nephrin
MEGERDRKAERERDLGEERKTEREEMERKRQREKLETDIERGTKRQTEADAGGRQWALGATGRGHGMALRIPVNAPLLLMGLLTTGLAQLPIPASAPRGFWALPENMTVVEGAAAELRCGVSAPGSAVQWAKDGLLLGPDRRIPGFPRYRLEGDPARGEFHLHIEACDLSDDAEYECQVSRSETGPELVSPRVILSVLVPPKVLQLTPEAGSTVTWVAGQEYEVSCVSGDAKPAPDITFVQSGQVIPDISANVNAGSQEKLFTTEAKVRVTPQSSDNGQLLVCEGSSPALDTPIKVSVTMNVLFPPGPPVIEWPGLDEGHVRAGQTLELLCMSRGGNPPATLQWLKNGQPLSTAWGTEHAHSVARSMLVMMVRPEDHGARLSCEAHNSVSTKIQERGVMLQVTFPPSAITILGSASQSENKNVTLSCITKSSRPRVLLRWWLGWRQLQPTEETVMDGLHGGHISMSNLTFLVRREDNGLTLTCEAFSDAFTKETFKKTLTLNVKYPAQKLWIEGPPVGQRLRAGTRVRLVCLAIGGNPDPTLTWYKDSRTVTEPRPPQEPRRVQLGSLEKSGSTFSRELVLVTGPSDNQAKFTCKAGQLSASTQFVVQFPPTNVTILANASALRPGEALNLTCVSVSSNPPVNLSWDKEGERLEGVAARARSAPFRGSAAARSVLLRMSSRDHGHRVTCRAHSAELRETVSAFYRLNVLYPPEFLGEQVLVVTAVEQGEALLPVSVSANPAPEAFNWTFRGYRLSPAGGPRHRILSGGALQLWNVTRADDGLYQLHCQNSEGTAEALVRLDVHYAPAIRALQDPTEVNVGGSVDIVCTVDANPILPGMFQWERLGEEEEDRSLDDMEMTSKGSTGRLQIRQAKLTQAGAYQCIADNGVAPPARGLVRLVVRFAPQVEHPTPLSKVAAAGDSTSSATLHCRARGVPNVVFTWTKNGVPLDLQDPRYTEHTYHQGGVHSSLLTIANVSAAQDYALFTCTATNPLGSDHINIQLVSISRPDPPSGLKVVSMTPYSVGLEWKPGFDGGLPQRFQIRYEALGTPGFLYVDVLPPQATTFTLTGLQPSTRYRVWLLASNALGDSGLADKGSQIPITTPGLDQPSGEPDYQLPTEQPAGPSELP

SEQ ID NO: 9 - protein, 1074 aa, synthetic construct
  source 1..1074: note = extracellular domain of sheep nephrin
EVGANTADIKDRGPGMALSTRIKAELLLLGLLTTGLTQVPILASAPRGFWALPENLTVVEGAVAELRCGVHAPGSAVQWAKDGLLLGPDPRIPSFPRYRLEGDHAKGEFHLRIEACDLSDDAEYECQVGRSETGPELVSPRVILSILVPPKVLQLTPEAGSTVTWVAGQEYTVSCVSGDAKPAPDITFLLSGQTISGISANVNEGSQQKLFTTEATARVTPQSSDNGQLLVCEGSSPALDTPIKASVTMNVLFPPGPPIIEWPGLDEGQVRAGQSLELSCTARGGNPLATLQWLKNGQPVSTAWGTEHAQAVARSLLVMIVRPEDHGARLSCEAYNSVSTGIQERGVTLQVTFPPSAITILGSASQSENKNVTVSCITKSSRPRVLLRWWLGWRQLQPSEETVMDGLHGGHISMSNLTFLARREDNGLTLTCEAFSEAFTKETFKKSLTLNVKYPAQKLWIEGPPEGQRLRAGNRVRLVCLAIGGNPDPSLTWYKASRTVTDPRPPQEPRRVQLGSVEKSGSIFSRELVLITGPSDNQAKFTCKAGQLSASTQLVVQFPPTNVTILANASTLRPGDALNLTCVSVSSNPPVNLSWDKEGERLEGVAAQPRRAPFKGSAAARSVLLRLSSRDHGHRVTCSAHSTELRETVSAFYRLNVLYPPEFLGEQVLVVTAVEQGEALLPVSVSPAPEAFNGTFRGYRLSPAGGPRHRILSGGALQLSNVTRADDGLYQLHCQNSEGTAEALVRLDVQYAPTIRALQDPTEVNVGDSVDIVCTVDANPILPEMFSWERLGEEGEDQSLDDMEKMSKGSTGRLRIHHAKLTQAGAYQCIVDNGVAPPARGLVRLVVRFAPHVEHPAPLTKVAAAGDSTSSATLHCRARGVPNIVFTWTKNGVPLDLQDPRYTEHTYHQGGVHSSLLTIANVSAAQDYALFTCIATNPLGSDHTNIQLVSISRPDPPSGLKAVSVTPYSVGLEWKPGFDGGLPQRFQIRYEALGTPGFLYMDVLPPQATSFTLTGLQPSTRYRVWLLASNALGDSGLVDKGSQISITTPGLDQPSREPDSQLPTEQPAGPSEMP

SEQ ID NO: 10 - protein, 1055 aa, synthetic construct
  source 1..1055: note = extracellular domain of goat nephrin
MALSTRIKAELLLLGLLTTGLTQVPILASAPRGFWALPENLTVVEGAIAELRCGVHAPGSAVQWAKDGLLLGPDPRIPSFPRYRLEGDPAKGEFHLHIEACDLSDDAEYECQVGRSETGPELVSPRVILSILVPPKVLQLTPEAGSTVTWVAGQEYTVSCVSGDAKPAPDITFLLSGQTISGISANVNEGSQQKLFTTEATARVTPQSSDNGQLLVCEGSSPALDTPIKASVTMNVLCKWRTELDEGQVRAGQSLELSCTARGGNPLATLQWLKNGQPVSTAWGTEHAQAVARSLLVMIVRPEDHGVRLSCEAYNSVSTGIQEHGVTLQVTFPPSAITILGSASQSENKNVTVSCITKSSRPRVLLRWWLGWRQLQPSEETVMDGLHGGHISMSNLTFLARREDNGLTLTCEAFSEAFTKETFKKSLTLNVKYPAQKLWIEGPPEGQRLRAGNRVRLVCLAIGGNPDPSLTWYKDSRTVTEPRPPQEPRRVQLGSVEKSGSIFSRELVLITGPSDNQAKFTCKAGQLSASTQLVVQFPPTNVTILANASTLRPGDALNLTCVSVSSNPPVNLSWDKEGERLEGVAAQPRRAPFKGSAAARSVLLRLSSRDHGHRVTCSAHSTELRETVSAFYRLNVLYPPEFLGEQVLVVTAVEQGEALLPVSVSANPAPEAFNWTFRGYRLSPAGGPRHRILSGGALQLWNVTRADDGLYQLHCQNSEGTAEALVRLDVQYAPTVRALQDPTEVNVGASVDIVCTVDANPILPEMFTWERLGEEGEDQSLDDMEKMSKGSTGRLRIHHAKLTQAGAYQCIVDNGVAPPARGLVRLVVRFAPHVEHPAPLTKVAAAGDSTSSATLHCRARGVPNIVFTWTKNGVPLDLQDPRYTEHTYHQGGVHSSLLTITNVSAAQDYALFTCIATNPLGSDHTNIQLVSISRPDPPSGLKAVSMTPYSVGLEWKPGFDGGLPQRFQIRYEALGTPGFLYMDVLPPQATTFTLTGLQPSTRYRVWLLASNALGDSGLVDKGSQISITTPGLDQPSREPDYQLPTEQPAGPSEMP

SEQ ID NO: 11 - protein, 1092 aa, synthetic construct
  source 1..1092: note = extracellular domain of camel nephrin
MRPRERDPERGRGRNRRQEVGPEGATGRGPGMAPRIPIMAPLLLMELLMTGLAQVPIPASAPRGFWALPENLTVVEGAAAELRCGVSSPGSAVQWAKDGLLLGPDPRIPGFPRYHLEGDPTRGEFHLRIEECDLSDDAEYECQVGRSETGPELVSPRVILSVLVPPKVLQLTPEAGSTVTWVAGQEYTVSCVSGDAKPAPDIAFLQRGKTISDISANVNEGSREKLFTTEATARVTPQSSDNGQLLVCEASSPALETPIKVSVTMNILFPPGPPVIEWPGLDEGHVRAGQSLELLCTARGGNPPATLQWLKNGQPVSTAWGTEHAQAVARSLLVMIVRPEDHGARLSCEAHNSVSTGIQERGVTLQVTFPPSAVTILGSASQSENKNVTLSCITKSSRPRVLLRWWLGWRQLLPTEETVMDGLYGGHISMSNLTFLARREDNGLTLTCEAFSEAFTKETFKKSLTLNVKYPAQKLWIEGPPEGQHLRAGTRVRLVCLAIGGNPDPSLIWYKDSRTVTEPRSPQEPRRVQLGSLEKSGSTFSRELVLVTGPSDNRAKFTCKAGQLSASTQLVVQFPPTNVTILANASALRPGDALNLTCVSVSSNPPVSLSWDKEGERLESVAARPQSAPFKGSAAARTVLLRMSPRDHGHRVTCRAHSTKLQETVSAFYRLNVLYPPEFLGEQVLVVTAVEKGEALLPVSVSANPAPEAFNWTFRGYRLSPAGGPRHRILSGGALQLWNVTRADDGLYQLHCQNSEGTAEALVRLDVHYAPTIRALQDPTEVNIGGSVDIVCTVDANPILPEMFNWERLGEEVEDQSLDDMEKMSKGSTGRLRIHHAKLTQAGAYQCIVDNGVAPPARGLVRLVVRFAPHVEHPAPLTKVAAAGDSTSSATLHCRARGVPNIVFTWSKNGVPLDLQDPRYTEHTYHQGGIHSSLLTIANVSAAQDYALFTCTATNPLGSDHTNIQLVSISRPDPPSGLKVMSMTPNSVGLEWKPGFDGGLPQSFRIRYEALGTPGFLYMDVLPPQATTFTLTGLQPSTRYRVWLLASNALGDSGLADKGSQISITTPGLDQPSGEPNYQLPTEQPAGPSELP

SEQ ID NO: 12 - protein, 1065 aa, synthetic construct
  source 1..1065: note = pre-Nephrin(ec)[human]-His
MALGTTLRASLLLLGLLTEGLAQLAIPASVPRGFWALPENLTVVEGASVELRCGVSTPGSAVQWAKDGLLLGPDPRIPGFPRYRLEGDPARGEFHLHIEACDLSDDAEYECQVGRSEMGPELVSPRVILSILVPPKLLLLTPEAGTMVTWVAGQEYVVNCVSGDAKPAPDITILLSGQTISDISANVNEGSQQKLFTVEATARVTPRSSDNRQLLVCEASSPALEAPIKASFTVNVLFPPGPPVIEWPGLDEGHVRAGQSLELPCVARGGNPLATLQWLKNGQPVSTAWGTEHTQAVARSVLVMTVRPEDHGAQLSCEAHNSVSAGTQEHGITLQVTFPPSAIIILGSASQTENKNVTLSCVSKSSRPRVLLRWWLGWRQLLPMEETVMDGLHGGHISMSNLTFLARREDNGLTLTCEAFSEAFTKETFKKSLILNVKYPAQKLWIEGPPEGQKLRAGTRVRLVCLAIGGNPEPSLMWYKDSRTVTESRLPQESRRVHLGSVEKSGSTFSRELVLVTGPSDNQAKFTCKAGQLSASTQLAVQFPPTNVTILANASALRPGDALNLTCVSVSSNPPVNLSWDKEGERLEGVAAPPRRAPFKGSAAARSVLLQVSSRDHGQRVTCRAHSAELRETVSSFYRLNVLYRPEFLGEQVLVVTAVEQGEALLPVSVSANPAPEAFNWTFRGYRLSPAGGPRHRILSSGALHLWNVTRADDGLYQLHCQNSEGTAEARLRLDVHYAPTIRALQDPTEVNVGGSVDIVCTVDANPILPGMFNWERLGEDEEDQSLDDMEKISRGPTGRLRIHHAKLAQAGAYQCIVDNGVAPPARRLLRLVVRFAPQVEHPTPLTKVAAAGDSTSSATLHCRARGVPNIVFTWTKNGVPLDLQDPRYTEHTYHQGGVHSSLLTIANVSAAQDYALFTCTATNALGSDQTNIQLVSISRPDPPSGLKVVSLTPHSVGLEWKPGFDGGLPQRFCIRYEALGTPGFHYVDVVPPQATTFTLTGLQPSTRYRVWLLASNALGDSGLADKGTQLPITTPGLHQPSGEPEDQLPTEPPSLEHHHHHHHH

SEQ ID NO: 13 - protein, 1088 aa, synthetic construct
  source 1..1088: note = pre-Nephrin(ec)[human]-H8-avi-b
MALGTTLRASLLLLGLLTEGLAQLAIPASVPRGFWALPENLTVVEGASVELRCGVSTPGSAVQWAKDGLLLGPDPRIPGFPRYRLEGDPARGEFHLHIEACDLSDDAEYECQVGRSEMGPELVSPRVILSILVPPKLLLLTPEAGTMVTWVAGQEYVVNCVSGDAKPAPDITILLSGQTISDISANVNEGSQQKLFTVEATARVTPRSSDNRQLLVCEASSPALEAPIKASFTVNVLFPPGPPVIEWPGLDEGHVRAGQSLELPCVARGGNPLATLQWLKNGQPVSTAWGTEHTQAVARSVLVMTVRPEDHGAQLSCEAHNSVSAGTQEHGITLQVTFPPSAIIILGSASQTENKNVTLSCVSKSSRPRVLLRWWLGWRQLLPMEETVMDGLHGGHISMSNLTFLARREDNGLTLTCEAFSEAFTKETFKKSLILNVKYPAQKLWIEGPPEGQKLRAGTRVRLVCLAIGGNPEPSLMWYKDSRTVTESRLPQESRRVHLGSVEKSGSTFSRELVLVTGPSDNQAKFTCKAGQLSASTQLAVQFPPTNVTILANASALRPGDALNLTCVSVSSNPPVNLSWDKEGERLEGVAAPPRRAPFKGSAAARSVLLQVSSRDHGQRVTCRAHSAELRETVSSFYRLNVLYRPEFLGEQVLVVTAVEQGEALLPVSVSANPAPEAFNWTFRGYRLSPAGGPRHRILSSGALHLWNVTRADDGLYQLHCQNSEGTAEARLRLDVHYAPTIRALQDPTEVNVGGSVDIVCTVDANPILPGMFNWERLGEDEEDQSLDDMEKISRGPTGRLRIHHAKLAQAGAYQCIVDNGVAPPARRLLRLVVRFAPQVEHPTPLTKVAAAGDSTSSATLHCRARGVPNIVFTWTKNGVPLDLQDPRYTEHTYHQGGVHSSLLTIANVSAAQDYALFTCTATNALGSDQTNIQLVSISRPDPPSGLKVVSLTPHSVGLEWKPGFDGGLPQRFCIRYEALGTPGFHYVDVVPPQATTFTLTGLQPSTRYRVWLLASNALGDSGLADKGTQLPITTPGLHQPSGEPEDQLPTEPPSLEGSGSGSHHHHHHHHGSGLNDIFEAQKIEWHE

SEQ ID NO: 14 - protein, 1241 aa, Homo sapiens
  source 1..1241: note = pre-Nephrin[human]
MALGTTLRASLLLLGLLTEGLAQLAIPASVPRGFWALPENLTVVEGASVELRCGVSTPGSAVQWAKDGLLLGPDPRIPGFPRYRLEGDPARGEFHLHIEACDLSDDAEYECQVGRSEMGPELVSPRVILSILVPPKLLLLTPEAGTMVTWVAGQEYVVNCVSGDAKPAPDITILLSGQTISDISANVNEGSQQKLFTVEATARVTPRSSDNRQLLVCEASSPALEAPIKASFTVNVLFPPGPPVIEWPGLDEGHVRAGQSLELPCVARGGNPLATLQWLKNGQPVSTAWGTEHTQAVARSVLVMTVRPEDHGAQLSCEAHNSVSAGTQEHGITLQVTFPPSAIIILGSASQTENKNVTLSCVSKSSRPRVLLRWWLGWRQLLPMEETVMDGLHGGHISMSNLTFLARREDNGLTLTCEAFSEAFTKETFKKSLILNVKYPAQKLWIEGPPEGQKLRAGTRVRLVCLAIGGNPEPSLMWYKDSRTVTESRLPQESRRVHLGSVEKSGSTFSRELVLVTGPSDNQAKFTCKAGQLSASTQLAVQFPPTNVTILANASALRPGDALNLTCVSVSSNPPVNLSWDKEGERLEGVAAPPRRAPFKGSAAARSVLLQVSSRDHGQRVTCRAHSAELRETVSSFYRLNVLYRPEFLGEQVLVVTAVEQGEALLPVSVSANPAPEAFNWTFRGYRLSPAGGPRHRILSSGALHLWNVTRADDGLYQLHCQNSEGTAEARLRLDVHYAPTIRALQDPTEVNVGGSVDIVCTVDANPILPGMFNWERLGEDEEDQSLDDMEKISRGPTGRLRIHHAKLAQAGAYQCIVDNGVAPPARRLLRLVVRFAPQVEHPTPLTKVAAAGDSTSSATLHCRARGVPNIVFTWTKNGVPLDLQDPRYTEHTYHQGGVHSSLLTIANVSAAQDYALFTCTATNALGSDQTNIQLVSISRPDPPSGLKVVSLTPHSVGLEWKPGFDGGLPQRFCIRYEALGTPGFHYVDVVPPQATTFTLTGLQPSTRYRVWLLASNALGDSGLADKGTQLPITTPGLHQPSGEPEDQLPTEPPSGPSGLPLLPVLFALGGLLLLSNASCVGGVLWQRRLRRLAEGISEKTEAGSEEDRVRNEYEESQWTGERDTQSSTVSTTEAEPYYRSLRDFSPQLPPTQEEVSYSRGFTGEDEDMAFPGHLYDEVERTYPPSGAWGPLYDEVQMGPWDLHWPEDTYQDPRGIYDQVAGDLDTLEPDSLPFELRGHLV

SEQ ID NO: 15 - protein, 353 aa, Homo sapiens
ASPTSPKVFPLSLCSTQPDGNVVIACLVQGFFPQEPLSVTWSESGQGVTARNFPPSQDASGDLYTTSSQLTLPATQCLAGKSVTCHVKHYTNPSQDVTVPCPVPSTPPTPSPSTPPTPSPSCCHPRLSLHRPALEDLLLGSEANLTCTLTGLRDASGVTFTWTPSSGKSAVQGPPERDLCGCYSVSSVLPGCAEPWNHGKTFTCTAAYPESKTPLTATLSKSGNTFRPEVHLLPPPSEELALNELVTLTCLARGFSPKDVLVRWLQGSQELPREKYLTWASRQEPSQGTTTFAVTSILRVAAEDWKKGDTFSCMVGHEALPLAFTQKTIDRLAGKPTHVNVSVVMAEVDGTCY

SEQ ID NO: 16 - protein, 340 aa, Homo sapiens
ASPTSPKVFPLSLDSTPQDGNVVVACLVQGFFPQEPLSVTWSESGQNVTARNFPPSQDASGDLYTTSSQLTLPATQCPDGKSVTCHVKHYTNSSQDVTVPCRVPPPPPCCHPRLSLHRPALEDLLLGSEANLTCTLTGLRDASGATFTWTPSSGKSAVQGPPERDLCGCYSVSSVLPGCAQPWNHGETFTCTAAHPELKTPLTANITKSGNTFRPEVHLLPPPSEELALNELVTLTCLARGFSPKDVLVRWLQGSQELPREKYLTWASRQEPSQGTTTYAVTSILRVAAEDWKKGETFSCMVGHEALPLAFTQKTIDRMAGKPTHINVSVVMAEADGTCY

SEQ ID NO: 17 - protein, 384 aa, Homo sapiens
APTKAPDVFPIISGCRHPKDNSPVVLACLITGYHPTSVTVTWYMGTQSQPQRTFPEIQRRDSYYMTSSQLSTPLQQWRQGEYKCVVQHTASKSKKEIFRWPESPKAQASSVPTAQPQAEGSLAKATTAPATTRNTGRGGEEKKKEKEKEEQEERETKTPECPSHTQPLGVYLLTPAVQDLWLRDKATFTCFVVGSDLKDAHLTWEVAGKVPTGGVEEGLLERHSNGSQSQHSRLTLPRSLWNAGTSVTCTLNHPSLPPQRLMALREPAAQAPVKLSLNLLASSDPPEAASWLLCEVSGFSPPNILLMWLEDQREVNTSGFAPARPPPQPRSTTFWAWSVLRVPAPPSPQPATYTCVVSHEDSRTLLNASRSLEVSYVTDHGPMK

SEQ ID NO: 18 - protein, 428 aa, Homo sapiens
ASTQSPSVFPLTRCCKNIPSNATSVTLGCLATGYFPEPVMVTWDTGSLNGTTMTLPATTLTLSGHYATISLLTVSGAWAKQMFTCRVAHTPSSTDWVDNKTFSVCSRDFTPPTVKILQSSCDGGGHFPPTIQLLCLVSGYTPGTINITWLEDGQVMDVDLSTASTTQEGELASTQSELTLSQKHWLSDRTYTCQVTYQGHTFEDSTKKCADSNPRGVSAYLSRPSPFDLFIRKSPTITCLVVDLAPSKGTVNLTWSRASGKPVNHSTRKEEKQRNGTLTVTSTLPVGTRDWIEGETYQCRVTHPHLPRALMRSTTKTSGPRAAPEVYAFATPEWPGSRDKRTLACLIQNFMPEDISVQWLHNEVQLPDARHSTTQPRKTKGSGFFVFSRLEVTRAEWEQKDEFICRAVHEAASPSQTVQRAVSVNPGK

SEQ ID NO: 19 - protein, 330 aa, Homo sapiens [sequence omitted]

SEQ ID NO: 20 - protein, 326 aa, Homo sapiens
ASTKGPSVFPLAPCSRSTSESTAALGCLVKDYFPEPVTVSWNSGALTSGVHTFPAVLQSSGLYSLSSVVTVPSSNFGTQTYTCNVDHKPSNTKVDKTVERKCCVECPPCPAPPVAGPSVFLFPPKPKDTLMISRTPEVTCVVVDVSHEDPEVQFNWYVDGVEVHNAKTKPREEQFNSTFRVVSVLTVVHQDWLNGKEYKCKVSNKGLPAPIEKTISKTKGQPREPQVYTLPPSREEMTKNQVSLTCLVKGFYPSDISVEWESNGQPENNYKTTPPMLDSDGSFFLYSKLTVDKSRWQQGNVFSCSVMHEALHNHYTQKSLSLSPGK

SEQ ID NO: 21 - protein, 377 aa, Homo sapiens
ASTKGPSVFPLAPCSRSTSGGTAALGCLVKDYFPEPVTVSWNSGALTSGVHTFPAVLQSSGLYSLSSVVTVPSSSLGTQTYTCNVNHKPSNTKVDKRVELKTPLGDTTHTCPRCPEPKSCDTPPPCPRCPEPKSCDTPPPCPRCPEPKSCDTPPPCPRCPAPELLGGPSVFLFPPKPKDTLMISRTPEVTCVVVDVSHEDPEVQFKWYVDGVEVHNAKTKPREEQYNSTFRVVSVLTVLHQDWLNGKEYKCKVSNKALPAPIEKTISKTKGQPREPQVYTLPPSREEMTKNQVSLTCLVKGFYPSDIAVEWESSGQPENNYNTTPPMLDSDGSFFLYSKLTVDKSRWQQGNIFSCSVMHEALHNRFTQKSLSLSPGK

SEQ ID NO: 22 - protein, 327 aa, Homo sapiens
ASTKGPSVFPLAPCSRSTSESTAALGCLVKDYFPEPVTVSWNSGALTSGVHTFPAVLQSSGLYSLSSVVTVPSSSLGTKTYTCNVDHKPSNTKVDKRVESKYGPPCPSCPAPEFLGGPSVFLFPPKPKDTLMISRTPEVTCVVVDVSQEDPEVQFNWYVDGVEVHNAKTKPREEQFNSTYRVVSVLTVLHQDWLNGKEYKCKVSNKGLPSSIEKTISKAKGQPREPQVYTLPPSQEEMTKNQVSLTCLVKGFYPSDIAVEWESNGQPENNYKTTPPVLDSDGSFFLYSRLTVDKSRWQEGNVFSCSVMHEALHNHYTQKSLSLSLGK

SEQ ID NO: 23 - protein, 453 aa, Homo sapiens
GSASAPTLFPLVSCENSPSDTSSVAVGCLAQDFLPDSITFSWKYKNNSDISSTRGFPSVLRGGKYAATSQVLLPSKDVMQGTDEHVVCKVQHPNGNKEKNVPLPVIAELPPKVSVFVPPRDGFFGNPRKSKLICQATGFSPRQIQVSWLREGKQVGSGVTTDQVQAEAKESGPTTYKVTSTLTIKESDWLGQSMFTCRVDHRGLTFQQNASSMCVPDQDTAIRVFAIPPSFASIFLTKSTKLTCLVTDLTTYDSVTISWTRQNGEAVKTHTNISESHPNATFSAVGEASICEDDWNSGERFTCTVTHTDLPSPLKQTISRPKGVALHRPDVYLLPPAREQLNLRESATITCLVTGFSPADVFVQWMQRGQPLSPEKYVTSAPMPEPQAPGRYFAHSILTVSEEEWNTGETYTCVVAHEALPNRVTERTVDKSTGKPTLYNVSLVMSDTAGTCY

SEQ ID NO: 24 - protein, 106 aa, Homo sapiens
GQPKANPTVTLFPPSSEELQANKATLVCLISDFYPGAVTVAWKADGSPVKAGVETTKPSKQSNNKYAASSYLSLTPEQWKSHRSYSCQVTHEGSTVEKTVAPTECS

SEQ ID NO: 25 - protein, 106 aa, Homo sapiens
GQPKAAPSVTLFPPSSEELQANKATLVCLISDFYPGAVTVAWKADSSPVKAGVETTTPSKQSNNKYAASSYLSLTPEQWKSHRSYSCQVTHEGSTVEKTVAPTECS

SEQ ID NO: 26 - protein, 106 aa, Homo sapiens
GQPKAAPSVTLFPPSSEELQANKATLVCLISDFYPGAVTVAWKADSSPVKAGVETTTPSKQSNNKYAASSYLSLTPEQWKSHKSYSCQVTHEGSTVEKTVAPTECS

SEQ ID NO: 27 - protein, 106 aa, Homo sapiens
GQPKAAPSVTLFPPSSEELQANKATLVCLISDFYPGAVKVAWKADGSPVNTGVETTTPSKQSNNKYAASSYLSLTPEQWKSHRSYSCQVTHEGSTVEKTVAPAECS

SEQ ID NO: 28 - protein, 106 aa, Homo sapiens
GQPKAAPSVTLFPPSSEELQANKATLVCLVSDFNPGAVTVAWKADGSPVKVGVETTKPSKQSNNKYAASSYLSLTPEQWKSHRSYSCRVTHEGSTVEKTVAPAECS

SEQ ID NO: 29 - protein, 107 aa, Homo sapiens [sequence omitted]